European Patent Specification EP 3 325 503 B1, published June 24, 2026. Title: Neuroprotective agents derived from spider venom peptides. Applicant: The University of Queensland. The sequence listing filed with the application follows.

SEQUENCE LISTING (35 sequences)

SEQ ID NO: 1 - DNA, 390 bp, Hadronyche infensa
atgaaatttccaaacttcgaagtaatgcttcttctggtgtggtctttaacgctttatgcagttggtgatgcaaaatatgaagatttattgaaaaatgctttagatgcaaagttattgaatgcatttgtggaaacgattcaattaaaaagccatgggaagagaaatgagtgcataaggaaatggttgtcttgtgttgatcggaaaaatgattgctgtgaggggctcgaatgctataagaggcgacattcgttcgaagtatgtgtacccattccgggattctgcttagtaaagtggaagcaatgcgatggacgagaacgggattgctgcgcaggtcttgaatgctggaagaggagtggaaataagtcctcagtctgtgcaccgattacatga

SEQ ID NO: 2 - protein, 129 aa, Hadronyche infensa
MKFPNFEVMLLLVWSLTLYAVGDAKYEDLLKNALDAKLLNAFVETIQLKSHGKRNECIRKWLSCVDRKNDCCEGLECYKRRHSFEVCVPIPGFCLVKWKQCDGRERDCCAGLECWKRSGNKSSVCAPIT

SEQ ID NO: 3 - DNA, 390 bp, Hadronyche infensa
atgaaatttccaaacttcgaagtaatgcttcttctggtgtggtctttaacgctttatgcagttggtgatgcaaaatatgaagatttattgaaaaatgctttagatgcaaagttatcgaatgcatttgtggaaacgattcaattaaaaagccatgggaagagaaatgagtgcataaggaaatggttgtcttgtgttgatcggaagaatgattgctgtgaggggctcgaatgctataagaggcgacattcgttcgaagtatgtgtacccattccgggattctgcttagtaaagtggaagcaatgcgatggacgagaacgggattgctgcccaggtcttgaatgctggaagaggagtggaaataagtcctcagtctgtgcaccaattacatga

SEQ ID NO: 4 - protein, 129 aa, Hadronyche infensa
MKFPNFEVMLLLVWSLTLYAVGDAKYEDLLKNALDAKLSNAFVETIQLKSHGKRNECIRKWLSCVDRKNDCCEGLECYKRRHSFEVCVPIPGFCLVKWKQCDGRERDCCPGLECWKRSGNKSSVCAPIT

SEQ ID NO: 5 - DNA, 456 bp, Hadronyche infensa
atgaaactcaggatcacgcttgctctgacatctgtgctggcattttgcgtctttggagataaagaaaatgaaaatttaatggaaaatcttttggaagacgacctattggatattttcacggacgctattcatatggaacgccaagaaacaaatcaggagtgcatagcgaaatggaaatcatgcgctggcagaaaactggattgttgtgaaggtcttgagtgctggaagaggagatggggacatgaagtgtgcgttccaattacacaaaagattttactgtttagaaaagtggaaaagtcatgttttgagaggaaatatgattgctgtgaagaacttgaatgctgggagaggagaggaaataagacacccagtatgcgcaccaaagcagtaaggtcagtcagtggtcatgaggctctcagtgttgcgctcctcaaaacttgtatacattacaaataa

SEQ ID NO: 6 - protein, 151 aa, Hadronyche infensa
MKLRITLALTSVLAFCVFGDKENENLMENLLEDDLLDIFTDAIHMERQETNQECIAKWKSCAGRKLDCCEGLECWKRRWGHEVCVPITQKILLFRKVEKSCFERKYDCCEELECWERRGNKTPSMRTKAVRSVSGHEALSVALLKTCIHYK

SEQ ID NO: 7 - DNA, 387 bp, Hadronyche infensa
atgaaactcaggatcacgcttgctctgacatcgatgctggcattttgcgtctttggagataaagaaaaggaaaatttaatggaaaatcttttggaagacgacctattggatatattcacggacgctattcatatggaacgccaggaaacaaatcaggagtgcatagcgaaatggaaatcatgcgctggcagaaaactggattgttgtgaaggtcttgagtgctggaagaggagatggggacatgaagtgtgcgttccaattacacaaaagattttctgtttagaaaagtggaagtcatgttttgagaggaaatatgattgctgtgaagaacttgaatgctgggagaggagaggaaataagcacccagtatgcgcaccaaagcagtaa

SEQ ID NO: 8 - protein, 128 aa, Hadronyche infensa
MKLRITLALTSMLAFCVFGDKEKENLMENLLEDDLLDIFTDAIHMERQETNQECIAKWKSCAGRKLDCCEGLECWKRRWGHEVCVPITQKIFCLEKWKSCFERKYDCCEELECWERRGNKHPVCAPKQ

SEQ ID NO: 9 - DNA, 390 bp, Hadronyche infensa
atgaaatttccaaacttcgaagtaatgcttcttctggtgtggtctttaacgctttatgcagttggtgatgcaaaatatgaagatttattgaaaaatgctttagatgcaaagttatcgaatgcatttgtggaaacgattcaattaaaaagccatgggaagagaaatgagtgcataaggaaatggttgtcttgtgttgatcggaaaaatgattgctgtgaggggctcgaatgctataagaggcgacattcgttcgaagtatgtgtacccattccgggattctgcttagtaaagtggaagcaatgcgatggacgagaacgggattgctgcgcaggtcttgaatgctggaagaggagtggaaataagtcctcagtctgtgcaccaattgcatga

SEQ ID NO: 10 - protein, 129 aa, Hadronyche infensa
MKFPNFEVMLLLVWSLTLYAVGDAKYEDLLKNALDAKLSNAFVETIQLKSHGKRNECIRKWLSCVDRKNDCCEGLECYKRRHSFEVCVPIPGFCLVKWKQCDGRERDCCAGLECWKRSGNKSSVCAPIA

SEQ ID NO: 11 - DNA, 390 bp, Hadronyche infensa
atgaaatttccaaacttcgaagtaatgcttcttctggtgtggtctttaacgctttatgcagttggtgatgcaaaatatgaagatttattgaaaaatgctttagatgcaaagttatcgaatgcatttgtggaaacgattcaattaaaaagccatgggaagagaaatgagtgcataaggaaatggttgtcttgtgttgatcggaaraatgattgctgtgaggggctcgaatgctataagaggcgacattcgttcgaagtatgtgtacccattccgggattctgcttagtaaagtggaagcaatgcgatggacgagaacgggattgctgcgcaggtcttgaatgctggaagaggagtggaaataagtcctcagtctgtgcaccaattgcatga

SEQ ID NO: 12 - protein, 129 aa, Hadronyche infensa; identical to SEQ ID NO: 10

SEQ ID NO: 13 - DNA, 228 bp, Hadronyche infensa
agcaatgaatgcattcgtaaatggctgagctgcgttgatcgtaaaaatgattgttgtgaaggcctggaatgctataaacgtcgtcatagctttgaagtttgtgttccgattccgggtttttgtctggttaaatggaaacagtgtgatggtcgtgaacgtgattgctgtgccggtctggaatgttggaaacgtagcggtaataaaagcagcgtttgtgcaccgatcacc

SEQ ID NO: 14 - protein, 76 aa, Hadronyche infensa
SNECIRKWLSCVDRKNDCCEGLECYKRRHSFEVCVPIPGFCLVKWKQCDGRERDCCAGLECWKRSGNKSSVCAPIT

SEQ ID NO: 15 - protein, 40 aa, Psalmopeous cambridgei
EDCIPKWKGCVNRHGDCCEGLECWKRRRSFEVCVPKTPKT

SEQ ID NO: 16 - protein, 75 aa, Hadronyche infensa
NECIRKWLSCVDRKNDCCEGLECYKRRHSFEVCVPIPGFCLVKWKQCDGRERDCCAGLECWKRSGNKSSVCAPIT

SEQ ID NO: 17 - protein, 37 aa, Hadronyche infensa
NECIRKWLSCVDRKNDCCEGLECYKRRHSFEVCVPIP

SEQ ID NO: 18 - protein, 35 aa, Hadronyche infensa
NECIRKWLSCVDRKNDCCEGLECYKRRHSFEVCVP

SEQ ID NO: 19 - protein, 37 aa, Hadronyche infensa; identical to SEQ ID NO: 17

SEQ ID NO: 20 - protein, 38 aa, Hadronyche infensa
NECIRKWLSCVDRKNDCCEGLECYKRRHSFEVCVPIPG

SEQ ID NO: 21 - protein, 40 aa, Hadronyche infensa
IPGFCLVKWKQCDGRERDCCAGLECWKRSGNKSSVCAPIT

SEQ ID NO: 22 - protein, 76 aa, Hadronyche infensa
SNECIRKWKSCVDRKNDCCEGLECYKRRHSFEVCVPIPGFCLVKWKQCDGRERDCCAGLECWKRSGNKSSVCAPIT

SEQ ID NO: 23 - protein, 76 aa, Hadronyche infensa
SNECIRKWLSCVDRKNDCCEGLECWKRRHSFEVCVPIPGFCLVKWKQCDGRERDCCAGLECWKRSGNKSSVCAPIT

SEQ ID NO: 24 - protein, 76 aa, Hadronyche infensa
SNECIRKWLSCVDRKNDCCEGLECYKRRRSFEVCVPIPGFCLVKWKQCDGRERDCCAGLECWKRSGNKSSVCAPIT

SEQ ID NO: 25 - protein, 78 aa, Engineered peptide
SEDCIPKWKGCVNRHGDCCEGLECWKRRRSFEVCVPKTEDCIPKWKGCVNRHGDCCEGLECWKRRRSFEVCVPKTPKT

SEQ ID NO: 26 - protein, 78 aa, Engineered peptide
SEDCIPKWKGCVNRHGDCCEGLECWKRRRSFEVCVPKTGDCIPKWKGCVNRHGDCCEGLECWKRRRSFEVCVPKTPKT

SEQ ID NO: 27 - protein, 79 aa, Engineered peptide
SNECIRKWLSCVDRKNDCCEGLECYKRRHSFEVCVPGGGGGGFCLVKWKQCDGRERDCCAGLECWKRSGNKSSVCAPIT

SEQ ID NO: 28 - protein, 81 aa, Engineered peptide
SEDCIPKWKGCVNRHGDCCEGLECWKRRRSFEVCVPKTPKTIPGFCLVKWKQCDGRERDCCAGLECWKRSGNKSSVCAPIT

SEQ ID NO: 29 - protein, 75 aa, Hadronyche infensa
NECIRKWLSCVDRKNDCCEGLECYKRRHSFEVCVPIPGFCLVKWKQCDGRERDCCPGLECWKRSGNKSSVCAPIT

SEQ ID NO: 30 - protein, 100 aa, Hadronyche infensa
QECIAKWKSCAGRKLDCCEGLECWKRRWGHEVCVPITQKILLFRKVEKSCFERKYDCCEELECWERRGNKTPSMRTKAVRSVSGHEALSVALLKTCIHYK

SEQ ID NO: 31 - protein, 77 aa, Hadronyche infensa
QECIAKWKSCAGRKLDCCEGLECWKRRWGHEVCVPITQKIFCLEKWKSCFERKYDCCEELECWERRGNKHPVCAPKQ

SEQ ID NO: 32 - protein, 75 aa, Hadronyche infensa
NECIRKWLSCVDRKNDCCEGLECYKRRHSFEVCVPIPGFCLVKWKQCDGRERDCCAGLECWKRSGNKSSVCAPIA

SEQ ID NO: 33 - protein, 75 aa, Hadronyche infensa; identical to SEQ ID NO: 32

SEQ ID NO: 34 - DNA, 1416 bp, Artificial sequence
  Coding sequence for recombinant Hi1a
atgatgttttccgcctcggctctcgccaaaatccatcaccatcaccatcacgaagaaggtaaactggtaatctggattaacggcgataaaggctataacggtctcgctgaagtcggtaagaaattcgagaaagataccggaattaaagtcaccgttgagcatccggataaactggaagagaaattcccacaggttgcggcaactggcgatggccctgacattatcttctgggcacacgaccgctttggtggctacgctcaatctggcctgttggctgaaatcaccccggacaaagcgttccaggacaagctgtatccgtttacctgggatgccgtacgttacaacggcaagctgattgcttacccgatcgctgttgaagcgttatcgctgatttataacaaagatctgctgccgaacccgccaaaaacctgggaagagatcccggcgctggataaagaactgaaagcgaaaggtaagagcgcgctgatgttcaacctgcaagaaccgtacttcacctggccgctgattgctgctgacgggggttatgcgttcaagtatgaaaacggcaagtacgacattaaagacgtgggcgtggataacgctggcgcgaaagcgggtctgaccttcctggttgacctgattaaaaacaaacacatgaatgcagacaccgattactccatcgcagaagctgcctttaataaaggcgaaacagcgatgaccatcaacggcccgtgggcatggtccaacatcgacaccagcaaagtgaattatggtgtaacggtactgccgaccttcaagggtcaaccatccaaaccgttcgttggcgtgctgagcgcaggtattaacgccgccagtccgaacaaagagctggcaaaagagttcctcgaaaactatctgctgactgatgaaggtctggaagcggttaataaagacaaaccgctgggtgccgtagcgctgaagtcttacgaggaagagttggcgaaagatccacgtattgccgccaccatggaaaacgcccagaaaggtgaaatcatgccgaacatcccgcagatgtccgctttctggtatgccgtgcgtactgcggtgatcaacgccgccagcggtcgtcagactgtcgatgaagccctgaaagacgcgcagactgattacgatatcccaggtaccgaaaacctgtattttcagagcaatgaatgcattcgtaaatggctgagctgcgttgatcgtaaaaatgattgttgtgaaggcctggaatgctataaacgtcgtcatagctttgaagtttgtgttccgattccgggtttttgtctggttaaatggaaacagtgtgatggtcgtgaacgtgattgctgtgccggtctggaatgttggaaacgtagcggtaataaaagcagcgtttgtgcaccgatcacctaataa

SEQ ID NO: 35 - protein, 470 aa, Artificial sequence
  Full precursor for recombinant Hi1a
MMFSASALAKIHHHHHHEEGKLVIWINGDKGYNGLAEVGKKFEKDTGIKVTVEHPDKLEEKFPQVAATGDGPDIIFWAHDRFGGYAQSGLLAEITPDKAFQDKLYPFTWDAVRYNGKLIAYPIAVEALSLIYNKDLLPNPPKTWEEIPALDKELKAKGKSALMFNLQEPYFTWPLIAADGGYAFKYENGKYDIKDVGVDNAGAKAGLTFLVDLIKNKHMNADTDYSIAEAAFNKGETAMTINGPWAWSNIDTSKVNYGVTVLPTFKGQPSKPFVGVLSAGINAASPNKELAKEFLENYLLTDEGLEAVNKDKPLGAVALKSYEEELAKDPRIAATMENAQKGEIMPNIPQMSAFWYAVRTAVINAASGRQTVDEALKDAQTDYDIPGTENLYFQSNECIRKWLSCVDRKNDCCEGLECYKRRHSFEVCVPIPGFCLVKWKQCDGRERDCCAGLECWKRSGNKSSVCAPIT